European Patent Application EP 4 414 380 A2, published August 14, 2024. Title: Universal anti-CD22 CHIMERIC ANTIGEN RECEPTOR ENGINEERED IMMUNE CELLS. Applicant: Cellectis SA. The sequence listing filed with the application follows.

SEQUENCE LISTING (26 sequences)

SEQ ID NO: 1 - protein, 21 aa, homo sapiens
  REGION 1..21: note = CD8alpha signal peptide
MALPVTALLLPLALLLHAARP

SEQ ID NO: 2 - protein, 20 aa, homo sapiens
  REGION 1..20: note = signal peptide
METDTLLLWVLLLWVPGSTG

SEQ ID NO: 3 - protein, 16 aa, homo sapiens
  REGION 1..16: note = FcgRIIIa hinge
GLAVSTISSFFPPGYQ

SEQ ID NO: 4 - protein, 45 aa, homo sapiens
  REGION 1..45: note = CD8alpha hinge
TTTPAPRPPTPAPTIASQPLSLRPEACRPAAGGAVHTRGLDFACD

SEQ ID NO: 5 - protein, 231 aa, homo sapiens
  REGION 1..231: note = IgG1 hinge
EPKSPDKTHTCPPCPAPPVAGPSVFLFPPKPKDTLMIARTPEVTCVVVDVSHEDPEVKFNWYVDGVEVHNAKTKPREEQYNSTYRVVSVLTVLHQDWLNGKEYKCKVSNKALPAPIEKTISKAKGQPREPQVYTLPPSRDELTKNQVSLTCLVKGFYPSDIAVEWESNGQPENNYKTTPPVLDSDGSFFLYSKLTVDKSRWQQGNVFSCSVMHEALHNHYTQKSLSLSPGK

SEQ ID NO: 6 - protein, 24 aa, homo sapiens
  REGION 1..24: note = CD8alpha transmembrane domain
IYIWAPLAGTCGVLLLSLVITLYC

SEQ ID NO: 7 - protein, 27 aa, homo sapiens
  REGION 1..27: note = 41BB transmembrane domain
IISFFLALTSTALLFLLFFLTLRFSVV

SEQ ID NO: 8 - protein, 42 aa, homo sapiens
  REGION 1..42: note = Fragment of 4-1BB (residues 214-255)
KRGRKKLLYIFKQPFMRPVQTTQEEDGCSCRFPEEEEGGCEL

SEQ ID NO: 9 - protein, 112 aa, homo sapiens
  REGION 1..112: note = fragment of T-cell surface glycoprotein CD3 zeta chain
RVKFSRSADAPAYQQGQNQLYNELNLGRREEYDVLDKRRGRDPEMGGKPRRKNPQEGLYNELQKDKMAEAYSEIGMKGERRRGKGHDGLYQGLSTATKDTYDALHMQALPPR

SEQ ID NO: 10 - protein, 15 aa, synthetic construct
  REGION 1..15: note = G4Sx3 linker sequence
GGGGSGGGGSGGGGS

SEQ ID NO: 11 - DNA, 1532 bp, homo sapiens
  misc_feature 1..1532: note = UCART22
  source 1..1532: mol_type = unassigned DNA
tgatcctcttgtcccacagatatccagaaccctgaccctgccgtgtaccagctgagagaatggctctgcccgtcaccgctctgctgctgccactggccctgctgctgcacgcagcaagaccacaggtgcagctgcagcagagcggccctggcctggtgaagccaagccagacactgtccctgacctgcgccatcagcggcgattccgtgagctccaactccgccgcctggaattggatcaggcagtccccttctcggggcctggagtggctgggaaggacatactatcggtctaagtggtacaacgattatgccgtgtctgtgaagagcagaatcacaatcaaccctgacacctccaagaatcagttctctctgcagctgaatagcgtgacaccagaggacaccgccgtgtactattgcgccagggaggtgaccggcgacctggaggatgcctttgacatctggggccagggcacaatggtgaccgtgtctagcggaggaggaggatccggaggaggaggatctggcggcggcggcagcgatatccagatgacacagtccccatcctctctgagcgcctccgtgggcgacagagtgacaatcacctgtagggcctcccagaccatctggtcttacctgaactggtatcagcagaggcccggcaaggcccctaatctgctgatctacgcagcaagctccctgcagagcggagtgccatccagattctctggcaggggctccggcacagacttcaccctgaccatctctagcctgcaggccgaggacttcgccacctactattgccagcagtcttatagcatcccccagacatttggccagggcaccaagctggagatcaagaccacaaccccagcaccaaggccacctacacctgcaccaaccatcgcctctcagcccctgagcctgagacctgaggcatgtaggccagcagcaggaggagcagtccatacaaggggtctggattttgcatgcgacatctacatctgggcacctctggcaggaacatgtggcgtgctcctgctcagcctggtcatcaccctgtactgcaagagaggcaggaagaagctgctgtatatcttcaagcagcccttcatgcgccccgtgcagacaacccaggaggaggatggctgctcctgtaggttcccagaagaggaggagggaggatgtgagctgcgcgtgaagttttcccggtctgccgacgcacctgcataccagcagggccagaaccagctgtataacgagctgaatctgggccggagagaggagtacgatgtgctggacaagaggcgcggcagagatccagagatgggcggcaagccccggagaaagaaccctcaggagggcctgtacaatgagctgcagaaggataagatggccgaggcctattctgagatcggcatgaagggagagaggcgccggggcaagggacacgacggactgtaccagggactgagcacagccaccaaggatacctatgacgccctgcatatgcaggcactgcctccaaggtga

SEQ ID NO: 12 - protein, 124 aa, synthetic construct
  REGION 1..124: note = 971- heavy chain
QVQLQQSGPGLVKPSQTLSLTCAISGDSVSSNSAAWNWIRQSPSRGLEWLGRTYYRSKWYNDYAVSVKSRITINPDTSKNQFSLQLNSVTPEDTAVYYCAREVTGDLEDAFDIWGQGTMVTVSS

SEQ ID NO: 13 - protein, 107 aa, synthetic construct
  REGION 1..107: note = 971- light chain
DIQMTQSPSSLSASVGDRVTITCRASQTIWSYLNWYQQRPGKAPNLLIYAASSLQSGVPSRFSGRGSGTDFTLTISSLQAEDFATYYCQQSYSIPQTFGQGTKLEIK

SEQ ID NO: 14 - protein, 464 aa, synthetic construct
  REGION 1..464: note = 971-v1 polypeptide CAR sequence
QVQLQQSGGGLVKPGASLKLSCVTSGFTFRKFGMSWVRQTSDKRLEWVASISTGGYNTYYSDNVKGRFTISRENAKNTLYLQMSSLKSEDTALYYCTRGYSSTSYAMDYWGQGTTVTVGGGGSGGGGSGGGGSDIELTQSPASLSVATGEKVTIRCMTSTDIDDDMNWYQQKPGEPPKFLISEGNTLRPGVPSRFSSSGTGTDFVFTIENTLSEDVGDYYCLQSFNVPLTFGDGTKLEKALTTTPAPRPPTPAPTIASQPLSLRPEACRPAAGGAVHTRGLDFACDIYIWAPLAGTCGVLLLSLVITLYCKRGRKKLLYIFKQPFMRPVQTTQEEDGCSCRFPEEEEGGCELRVKFSRSADAPAYQQGQNQLYNELNLGRREEYDVLDKRRGRDPEMGGKPRRKNPQEGLYNELQKDKMAEAYSEIGMKGERRRGKGHDGLYQGLSTATKDTYDALHMQALPPR

SEQ ID NO: 15 - protein, 650 aa, synthetic construct
  REGION 1..650: note = 971-v3 polypeptide CAR sequence
QVQLQQSGGGLVKPGASLKLSCVTSGFTFRKFGMSWVRQTSDKRLEWVASISTGGYNTYYSDNVKGRFTISRENAKNTLYLQMSSLKSEDTALYYCTRGYSSTSYAMDYWGQGTTVTVGGGGSGGGGSGGGGSDIELTQSPASLSVATGEKVTIRCMTSTDIDDDMNWYQQKPGEPPKFLISEGNTLRPGVPSRFSSSGTGTDFVFTIENTLSEDVGDYYCLQSFNVPLTFGDGTKLEKALEPKSPDKTHTCPPCPAPPVAGPSVFLFPPKPKDTLMIARTPEVTCVVVDVSHEDPEVKFNWYVDGVEVHNAKTKPREEQYNSTYRVVSVLTVLHQDWLNGKEYKCKVSNKALPAPIEKTISKAKGQPREPQVYTLPPSRDELTKNQVSLTCLVKGFYPSDIAVEWESNGQPENNYKTTPPVLDSDGSFFLYSKLTVDKSRWQQGNVFSCSVMHEALHNHYTQKSLSLSPGKIYIWAPLAGTCGVLLLSLVITLYCKRGRKKLLYIFKQPFMRPVQTTQEEDGCSCRFPEEEEGGCELRVKFSRSADAPAYQQGQNQLYNELNLGRREEYDVLDKRRGRDPEMGGKPRRKNPQEGLYNELQKDKMAEAYSEIGMKGERRRGKGHDGLYQGLSTATKDTYDALHMQALPPR

SEQ ID NO: 16 - protein, 530 aa, synthetic construct
  REGION 1..530: note = TAL binding domain TRAC_T01-L
LTPQQVVAIASNGGGKQALETVQRLLPVLCQAHGLTPQQVVAIASNNGGKQALETVQRLLPVLCQAHGLTPQQVVAIASNGGGKQALETVQRLLPVLCQAHGLTPEQVVAIASHDGGKQALETVQRLLPVLCQAHGLTPEQVVAIASHDGGKQALETVQRLLPVLCQAHGLTPEQVVAIASHDGGKQALETVQRLLPVLCQAHGLTPEQVVAIASNIGGKQALETVQALLPVLCQAHGLTPEQVVAIASHDGGKQALETVQRLLPVLCQAHGLTPEQVVAIASNIGGKQALETVQALLPVLCQAHGLTPQQVVAIASNNGGKQALETVQRLLPVLCQAHGLTPEQVVAIASNIGGKQALETVQALLPVLCQAHGLTPQQVVAIASNGGGKQALETVQRLLPVLCQAHGLTPEQVVAIASNIGGKQALETVQALLPVLCQAHGLTPQQVVAIASNGGGKQALETVQRLLPVLCQAHGLTPEQVVAIASHDGGKQALETVQRLLPVLCQAHGLTPQQVVAIASNGGGRPALE

SEQ ID NO: 17 - protein, 530 aa, synthetic construct
  REGION 1..530: note = TAL binding domain TRAC_T01-R
LTPEQVVAIASHDGGKQALETVQRLLPVLCQAHGLTPQQVVAIASNGGGKQALETVQRLLPVLCQAHGLTPEQVVAIASHDGGKQALETVQRLLPVLCQAHGLTPEQVVAIASNIGGKQALETVQALLPVLCQAHGLTPQQVVAIASNNGGKQALETVQRLLPVLCQAHGLTPEQVVAIASHDGGKQALETVQRLLPVLCQAHGLTPQQVVAIASNGGGKQALETVQRLLPVLCQAHGLTPQQVVAIASNNGGKQALETVQRLLPVLCQAHGLTPQQVVAIASNNGGKQALETVQRLLPVLCQAHGLTPQQVVAIASNGGGKQALETVQRLLPVLCQAHGLTPEQVVAIASNIGGKQALETVQALLPVLCQAHGLTPEQVVAIASHDGGKQALETVQRLLPVLCQAHGLTPEQVVAIASNIGGKQALETVQALLPVLCQAHGLTPEQVVAIASHDGGKQALETVQRLLPVLCQAHGLTPQQVVAIASNNGGKQALETVQRLLPVLCQAHGLTPQQVVAIASNGGGRPALE

SEQ ID NO: 18 - DNA, 49 bp, synthetic construct
  misc_feature 1..49: note = target TALEN TRAC_T01
  source 1..49: mol_type = other DNA
ttgtcccacagatatccagaaccctgaccctgccgtgtaccagctgaga

SEQ ID NO: 19 - protein, 9 aa, synthetic construct
  REGION 1..9: note = Mimotope of CD20 antigen
CPYSNPSLC

SEQ ID NO: 20 - DNA, 1473 bp, synthetic construct
  misc_feature 1..1473: note = CAR 11 dis 16
  source 1..1473: mol_type = other DNA
atggctctgcccgtcaccgctctgctgctgccactggccctgctgctgcacgcagcaagaccacaggtgcagctgcagcagagcggccctggcctggtgaagccaagccagacactgtccctgacctgcgccatcagcggcgattccgtgagctccaactccgccgcctggaattggatcaggcagtccccttctcggggcctggagtggctgggaaggacatactatcggtctaagtggtacaacgattatgccgtgtctgtgaagagcagaatcacaatcaaccctgacacctccaagaatcagttctctctgcagctgaatagcgtgacaccagaggacaccgccgtgtactattgcgccagggaggtgaccggcgacctggaggatgcctttgacatctggggccagggcacaatggtgaccgtgtctagcggaggaggaggatccggaggaggaggatctggcggcggcggcagcgatatccagatgacacagtccccatcctctctgagcgcctccgtgggcgacagagtgacaatcacctgtagggcctcccagaccatctggtcttacctgaactggtatcagcagaggcccggcaaggcccctaatctgctgatctacgcagcaagctccctgcagagcggagtgccatccagattctctggcaggggctccggcacagacttcaccctgaccatctctagcctgcaggccgaggacttcgccacctactattgccagcagtcttatagcatcccccagacatttggccagggcaccaagctggagatcaagaccacaaccccagcaccaaggccacctacacctgcaccaaccatcgcctctcagcccctgagcctgagacctgaggcatgtaggccagcagcaggaggagcagtccatacaaggggtctggattttgcatgcgacatctacatctgggcacctctggcaggaacatgtggcgtgctcctgctcagcctggtcatcaccctgtactgcaagagaggcaggaagaagctgctgtatatcttcaagcagcccttcatgcgccccgtgcagacaacccaggaggaggatggctgctcctgtaggttcccagaagaggaggagggaggatgtgagctgcgcgtgaagttttcccggtctgccgacgcacctgcataccagcagggccagaaccagctgtataacgagctgaatctgggccggagagaggagtacgatgtgctggacaagaggcgcggcagagatccagagatgggcggcaagccccggagaaagaaccctcaggagggcctgtacaatgagctgcagaaggataagatggccgaggcctattctgagatcggcatgaagggagagaggcgccggggcaagggacacgacggactgtaccagggactgagcacagccaccaaggatacctatgacgccctgcatatgcaggcactgcctccaaggtga

SEQ ID NO: 21 - DNA, 59 bp, synthetic construct
  misc_feature 1..59: note = TARGET TALEN(R)
  source 1..59: mol_type = other DNA
tgatcctcttgtcccacagatatccagaaccctgaccctgccgtgtaccagctgagaga

SEQ ID NO: 22 - DNA, 1473 bp, synthetic construct; identical to SEQ ID NO: 20
  misc_feature 1..1473: note = 971-v3 polynucleotide CAR sequence
  source 1..1473: mol_type = other DNA

SEQ ID NO: 23 - protein, 489 aa, synthetic construct
  REGION 1..489: note = CAR distal CD22
MALPVTALLLPLALLLHAARPEVQLVESGGGLVKPGGSLKLSCAASGFAFSIYDMSWVRQTPEKRLEWVAYISSGGGTYYPDTVKGRFTISRDNAKNTLYLQMSSLKSEDTAMYYCARHSGYGTHWGVLFAYWGQGTLVTVSAGGGGSGGGGSGGGGSDIQMTQTTSSLSASLGDRVTISCRASQDISNYLNWYQQKPDGTVKLLIYYTSILHSGVPSRFSGSGSGTDYSLTISNLEQEDFATYFCQQGNTLPWTFGGGTKLEIKATTTPAPRPPTPAPTIASQPLSLRPEACRPAAGGAVHTRGLDFACDIYIWAPLAGTCGVLLLSLVITLYCKRGRKKLLYIFKQPFMRPVQTTQEEDGCSCRFPEEEEGGCELRVKFSRSADAPAYQQGQNQLYNELNLGRREEYDVLDKRRGRDPEMGGKPRRKNPQEGLYNELQKDKMAEAYSEIGMKGERRRGKGHDGLYQGLSTATKDTYDALHMQALPPR

SEQ ID NO: 24 - DNA, 1470 bp, synthetic construct
  misc_feature 1..1470: note = CAR distal CD22
  source 1..1470: mol_type = other DNA
atggctctgcccgtcaccgctctgctgctgccactggccctgctgctgcacgcagcaaggcctgaggtgcagctggtggaatccggaggaggcctggtgaagcctggcggctctctgaagctgagctgtgccgcctccggcttcgccttttccatctacgacatgtcttgggtgaggcagaccccagagaagcgcctggagtgggtggcctatatcagctccggcggcggcacctactatcccgacacagtgaagggccggttcaccatctctagagataacgccaagaatacactgtacctgcagatgtctagcctgaagagcgaggataccgccatgtactattgcgcaaggcactccggatacggaacacactggggcgtgctgtttgcctattggggccagggcaccctggtgacagtgagcgccggaggaggaggaagcggcggaggaggctccggcggcggcggctctgacatccagatgacccagaccacatcctctctgagcgcctccctgggcgacagggtgacaatctcttgtagagccagccaggatatctccaactacctgaattggtatcagcagaagcctgatggcaccgtgaagctgctgatctactatacatctatcctgcacagcggagtgccatcccggttctctggaagcggatccggaaccgactactctctgacaatcagcaacctggagcaggaggatttcgccacctatttttgccagcagggcaataccctgccttggacatttggcggcggcacaaagctggagatcaaggccaccacaacccctgcaccaaggccaccaacaccagcacctaccatcgcatctcagcctctgagcctgagaccagaggcatgtaggccagcagcaggaggagcagtgcacacaaggggactggattttgcctgtgatatctacatctgggcacctctggcaggaacatgtggcgtgctcctgctcagcctggtcatcaccctgtactgcaagagaggcaggaagaagctgctgtatatcttcaagcagcccttcatgagacccgtgcagacaacccaggaggaggacggctgctcctgtaggttcccagaagaggaggagggaggatgtgagctgcgcgtgaagttttcccggtctgccgatgcacctgcataccagcagggacagaatcagctgtataacgagctgaatctgggccggagagaggagtacgacgtgctggataagaggaggggaagggacccagagatgggaggcaagcctcggagaaagaacccacaggagggcctgtacaatgagctgcagaaggacaagatggccgaggcctattctgagatcggcatgaagggagagaggcgccggggcaagggacacgatggcctgtaccagggcctgtccacagccaccaaggacacctatgatgccctgcatatgcaggcactgcctccaaggtga

SEQ ID NO: 25 - protein, 495 aa, synthetic construct
  REGION 1..495: note = description of artificial sequence: synthetic polypeptide
  REGION 1..495: note = 4G7-CAR version 1
MALPVTALLLPLALLLHAARPEVQLQQSGPELIKPGASVKMSCKASGYTFTSYVMHWVKQKPGQGLEWIGYINPYNDGTKYNEKFKGKATLTSDKSSSTAYMELSSLTSEDSAVYYCARGTYYYGSRVFDYWGQGTTLTVSSGGGGSGGGGSGGGGSDIVMTQAAPSIPVTPGESVSISCRSSKSLLNSNGNTYLYWFLQRPGQSPQLLIYRMSNLASGVPDRFSGSGSGTAFTLRISRVEAEDVGVYYCMQHLEYPFTFGAGTKLELKRADTTTPAPRPPTPAPTIASQPLSLRPEACRPAAGGAVHTRGLDFACDIYIWAPLAGTCGVLLLSLVITLYCKRGRKKLLYIFKQPFMRPVQTTQEEDGCSCRFPEEEEGGCELRVKFSRSADAPAYQQGQNQLYNELNLGRREEYDVLDKRRGRDPEMGGKPRRKNPQEGLYNELQKDKMAEAYSEIGMKGERRRGKGHDGLYQGLSTATKDTYDALHMQALPPR

SEQ ID NO: 26 - protein, 495 aa, synthetic construct
  REGION 1..495: note = description of artificial sequence: synthetic polypeptide
  REGION 1..495: note = 4G7-CAR version 2
METDTLLLWVLLLWVPGSTGEVQLQQSGPELIKPGASVKMSCKASGYTFTSYVMHWVKQKPGQGLEWIGYINPYNDGTKYNEKFKGKATLTSDKSSSTAYMELSSLTSEDSAVYYCARGTYYYGSRVFDYWGQGTTLTVSSGGGGSGGGGSGGGGSDIVMTQAAPSIPVTPGESVSISCRSSKSLLNSNGNTYLYWFLQRPGQSPQLLIYRMSNLASGVPDRFSGSGSGTAFTLRISRVEAEDVGVYYCMQHLEYPFTFGAGTKLELKRSDPTTTPAPRPPTPAPTIASQPLSLRPEACRPAAGGAVHTRGLDFACDIYIWAPLAGTCGVLLLSLVITLYCKRGRKKLLYIFKQPFMRPVQTTQEEDGCSCRFPEEEEGGCELRVKFSRSADAPAYQQGQNQLYNELNLGRREEYDVLDKRRGRDPEMGGKPRRKNPQEGLYNELQKDKMAEAYSEIGMKGERRRGKGHDGLYQGLSTATKDTYDALHMQALPPR